European Patent Specification EP 3 592 839 B1, published July 5, 2023. Title: MR1 RESTRICTED T CELL RECEPTORS FOR CANCER IMMUNOTHERAPY. Applicant: Universität Basel. The sequence listing filed with the application follows.

SEQUENCE LISTING (58 sequences)

SEQ ID NO: 1 - protein, 267 aa, Homo sapiens
MWGVFLLYVSMKMGGTTGQNIDQPTEMTATEGAIVQINCTYQTSGFNGLFWYQQHAGEAPTFLSYNVLDGLEEKGRFSSFLSRSKGYSYLLLKELQMKDSASYLCAVMDSSYKLIFGSGTRLLVRPDIQNPDPAVYQLRDSKSSDKSVCLFTDFDSQTNVSQSKDSDVYITDKTVLDMRSMDFKSNSAVAWSNKSDFACANAFNNSIIPEDTFFPSPESSCDVKLVEKSFETDTNLNFQNLSVIGFRILLLKVAGFNLLMTLRLWSS

SEQ ID NO: 2 - protein, 271 aa, Homo sapiens
MLLITSMLVLWMQLSQVNGQQVMQIPQYQHVQEGEDFTTYCNSSTTLSNIQWYKQRPGGHPVFLIQLVKSGEVKKQKRLTFQFGEAKKNSSLHITATQTTDVGTYFCAAAGGTSYGKLTFGQGTILTVHPNIQNPDPAVYQLRDSKSSDKSVCLFTDFDSQTNVSQSKDSDVYITDKTVLDMRSMDFKSNSAVAWSNKSDFACANAFNNSIIPEDTFFPSPESSCDVKLVEKSFETDTNLNFQNLSVIGFRILLLKVAGFNLLMTLRLWSS

SEQ ID NO: 3 - protein, 277 aa, Homo sapiens
MKTFAGFSFLFLWLQLDCMSRGEDVEQSLFLSVREGDSSVINCTYTDSSSTYLYWYKQEPGAGLQLLTYIFSNMDMKQDQRLTVLLNKKDKHLSLRIADTQTGDSAIYFCAETWTDRGSTLGRLYFGRGTQLTVWPDIQNPDPAVYQLRDSKSSDKSVCLFTDFDSQTNVSQSKDSDVYITDKTVLDMRSMDFKSNSAVAWSNKSDFACANAFNNSIIPEDTFFPSPESSCDVKLVEKSFETDTNLNFQNLSVIGFRILLLKVAGFNLLMTLRLWSS

SEQ ID NO: 4 - protein, 280 aa, Homo sapiens
MAMLLGASVLILWLQTDWVNSQQKNDDQQVKQNSPSLSVQEGRISILNCDYTNSMFDYFLWYKKYPAEGPTFLISISSIKDKNEDGRFTVFLNKSAKHLSLHIVPSQPGDSAVYFCAASLYNQGGKLIFGQGTELSVKPNIQNPDPAVYQLRDSKSSDKSVCLFTDFDSQTNVSQSKDSDVYITDKTVLDMRSMDFKSNSAVAWSNKSDFACANAFNNSIIPEDTFFPSPESSCDVKLVEKSFETDTNLNFQNLSVIGFRILLLKVAGFNLLMTLRLWSS

SEQ ID NO: 5 - protein, 274 aa, Homo sapiens
MEKNPLAAPLLILWFHLDCVSSILNVEQSPQSLHVQEGDSTNFTCSFPSSNFYALHWYRWETAKSPEALFVMTLNGDEKKKGRISATLNTKEGYSYLYIKGSQPEDSATYLCASGDSGYALNFGKGTSLLVTPHIQNPDPAVYQLRDSKSSDKSVCLFTDFDSQTNVSQSKDSDVYITDKTVLDMRSMDFKSNSAVAWSNKSDFACANAFNNSIIPEDTFFPSPESSCDVKLVEKSFETDTNLNFQNLSVIGFRILLLKVAGFNLLMTLRLWSS

SEQ ID NO: 6 - protein, 276 aa, Homo sapiens
MNYSPGLVSLILLLLGRTRGNSVTQMEGPVTLSEEAFLTINCTYTATGYPSLFWYVQYPGEGLQLLLKATKADDKGSNKGFEATYRKETTSFHLEKGSVQVSDSAVYFCALTIWDYGGSQGNLIFGKGTKLSVKPNIQNPDPAVYQLRDSKSSDKSVCLFTDFDSQTNVSQSKDSDVYITDKTVLDMRSMDFKSNSAVAWSNKSDFACANAFNNSIIPEDTFFPSPESSCDVKLVEKSFETDTNLNFQNLSVIGFRILLLKVAGFNLLMTLRLWSS

SEQ ID NO: 7 - protein, 269 aa, Homo sapiens
MVLKFSVSILWIQLAWVSTQLLEQSPQFLSIQEGENLTVYCNSSSVFSSLQWYRQEPGEGPVLLVTVVTGGEVKKLKRLTFQFGDARKDSSLHITAAQPGDTGLYLCAGENSGYALNFGKGTSLLVTPHIQNPDPAVYQLRDSKSSDKSVCLFTDFDSQTNVSQSKDSDVYITDKTVLDMRSMDFKSNSAVAWSNKSDFACANAFNNSIIPEDTFFPSPESSCDVKLVEKSFETDTNLNFQNLSVIGFRILLLKVAGFNLLMTLRLWSS

SEQ ID NO: 8 - protein, 275 aa, Homo sapiens
MMKSLRVLLVILWLQLSWVWSQQKEVEQDPGPLSVPEGAIVSLNCTYSNSAFQYFMWYRQYSRKGPELLMYTYSSGNKEDGRFTAQVDKSSKYISLFIRDSQPSDSATYLCAMSLSGGSYIPTFGRGTSLIVHPYIQNPDPAVYQLRDSKSSDKSVCLFTDFDSQTNVSQSKDSDVYITDKTVLDMRSMDFKSNSAVAWSNKSDFACANAFNNSIIPEDTFFPSPESSCDVKLVEKSFETDTNLNFQNLSVIGFRILLLKVAGFNLLMTLRLWSS

SEQ ID NO: 9 - protein, 275 aa, Homo sapiens
MLLEHLLIILWMQLTWVSGQQLNQSPQSMFIQEGEDVSMNCTSSSIFNTWLWYKQDPGEGPVLLIALYKAGELTSNGRLTAQFGITRKDSFLNISASIPSDVGIYFCAGQLGGAGGTSYGKLTFGQGTILTVHPNIQNPDPAVYQLRDSKSSDKSVCLFTDFDSQTNVSQSKDSDVYITDKTVLDMRSMDFKSNSAVAWSNKSDFACANAFNNSIIPEDTFFPSPESSCDVKLVEKSFETDTNLNFQNLSVIGFRILLLKVAGFNLLMTLRLWSS

SEQ ID NO: 10 - protein, 274 aa, Homo sapiens
MTSIRAVFIFLWLQLDLVNGENVEQHPSTLSVQEGDSAVIKCTYSDSASNYFPWYKQELGKGPQLIIDIRSNVGEKKDQRIAVTLNKTAKHFSLHITETQPEDSAVYFCAANWSPQGNEKLTFGTGTRLTIIPNIQNPDPAVYQLRDSKSSDKSVCLFTDFDSQTNVSQSKDSDVYITDKTVLDMRSMDFKSNSAVAWSNKSDFACANAFNNSIIPEDTFFPSPESSCDVKLVEKSFETDTNLNFQNLSVIGFRILLLKVAGFNLLMTLRLWSS

SEQ ID NO: 11 - protein, 267 aa, Homo sapiens
MWGVFLLYVSMKMGGTTGQNIDQPTEMTATEGAIVQINCTYQTSGFNGLFWYQQHAGEAPTFLSYNVLDGLEEKGRFSSFLSRSKGYSYLLLKELQMKDSASYLCASMDSNYQLIWGAGTKLIIKPDIQNPDPAVYQLRDSKSSDKSVCLFTDFDSQTNVSQSKDSDVYITDKTVLDMRSMDFKSNSAVAWSNKSDFACANAFNNSIIPEDTFFPSPESSCDVKLVEKSFETDTNLNFQNLSVIGFRILLLKVAGFNLLMTLRLWSS

SEQ ID NO: 12 - protein, 274 aa, homo sapiens
MISLRVLLVILWLQLSWVWSQRKEVEQDPGPFNVPEGATVAFNCTYSNSASQSFFWYRQDCRKEPKLLMSVYSSGNEDGRFTAQLNRASQYISLLIRDSKLSDSATYLCVVNRFTRDGNKLVFGAGTILRVKSYIQNPDPAVYQLRDSKSSDKSVCLFTDFDSQTNVSQSKDSDVYITDKTVLDMRSMDFKSNSAVAWSNKSDFACANAFNNSIIPEDTFFPSPESSCDVKLVEKSFETDTNLNFQNLSVIGFRILLLKVAGFNLLMTLRLWSS

SEQ ID NO: 13 - protein, 314 aa, Homo sapiens
MLLLLLLLGPGSGLGAVVSQHPSWVICKSGTSVKIECRSLDFQATTMFWYRQFPKQSLMLMATSNEGSKATYEQGVEKDKFLINHASLTLSTLTVTSAHPEDSSFYICSAKVTSGQHQGTTDTQYFGPGTRLTVLEDLKNVFPPEVAVFEPSEAEISHTQKATLVCLATGFYPDHVELSWWVNGKEVHSGVSTDPQPLKEQPALNDSRYCLSSRLRVSATFWQNPRNHFRCQVQFYGLSENDEWTQDRAKPVTQIVSAEAWGRADCGFTSESYQQGVLSATILYEILLGKATLYAVLVSALVLMAMVKRKDSRG

SEQ ID NO: 14 - protein, 311 aa, Homo sapiens
MTIRLLCYMGFYFLGAGLMEADIYQTPRYLVIGTGKKITLECSQTMGHDKMYWYQQDPGMELHLIHYSYGVNSTEKGDLSSESTVSRIRTEHFPLTLESARPSHTSQYLCASSEYIQYSGNTIYFGEGSWLTVVEDLNKVFPPEVAVFEPSEAEISHTQKATLVCLATGFFPDHVELSWWVNGKEVHSGVSTDPQPLKEQPALNDSRYCLSSRLRVSATFWQNPRNHFRCQVQFYGLSENDEWTQDRAKPVTQIVSAEAWGRADCGFTSVSYQQGVLSATILYEILLGKATLYAVLVSALVLMAMVKRKDF

SEQ ID NO: 15 - protein, 312 aa, Homo sapiens
MGFRLLCCVAFCLLGAGPVDSGVTQTPKHLITATGQRVTLRCSPRSGDLSVYWYQQSLDQGLQFLIQYYNGEERAKGNILERFSAQQFPDLHSELNLSSLELGDSALYFCASSVGGGLADTQYFGPGTRLTVLEDLKNVFPPEVAVFEPSEAEISHTQKATLVCLATGFYPDHVELSWWVNGKEVHSGVSTDPQPLKEQPALNDSRYCLSSRLRVSATFWQNPRNHFRCQVQFYGLSENDEWTQDRAKPVTQIVSAEAWGRADCGFTSESYQQGVLSATILYEILLGKATLYAVLVSALVLMAMVKRKDSRG

SEQ ID NO: 16 - protein, 313 aa, Homo sapiens
MSIGLLCCAALSLLWAGPVNAGVTQTPKFQVLKTGQSMTLQCAQDMNHEYMSWYRQDPGMGLRLIHYSVGAGITDQGEVPNGYNVSRSTTEDFPLRLLSAAPSQTSVYFCASGISGTASSYNSPLHFGNGTRLTVTEDLNKVFPPEVAVFEPSEAEISHTQKATLVCLATGFFPDHVELSWWVNGKEVHSGVSTDPQPLKEQPALNDSRYCLSSRLRVSATFWQNPRNHFRCQVQFYGLSENDEWTQDRAKPVTQIVSAEAWGRADCGFTSVSYQQGVLSATILYEILLGKATLYAVLVSALVLMAMVKRKDF

SEQ ID NO: 17 - protein, 309 aa, Homo sapiens
MGPGLLHWMALCLLGTGHGDAMVIQNPRYQVTQFGKPVTLSCSQTLNHNVMYWYQQKSSQAPKLLFHYYDKDFNNEADTPDNFQSRRPNTSFCFLDIRSPGLGDAAMYLCATSREWETQYFGPGTRLLVLEDLKNVFPPEVAVFEPSEAEISHTQKATLVCLATGFYPDHVELSWWVNGKEVHSGVSTDPQPLKEQPALNDSRYCLSSRLRVSATFWQNPRNHFRCQVQFYGLSENDEWTQDRAKPVTQIVSAEAWGRADCGFTSESYQQGVLSATILYEILLGKATLYAVLVSALVLMAMVKRKDSRG

SEQ ID NO: 18 - protein, 315 aa, Homo sapiens
MTIRLLCYMGFYFLGAGLMEADIYQTPRYLVIGTGKKITLECSQTMGHDKMYWYQQDPGMELHLIHYSYGVNSTEKGDLSSESTVSRIRTEHFPLTLESARPSHTSQYLCASSQLYRDTSNTGELFFGEGSRLTVLEDLKNVFPPEVAVFEPSEAEISHTQKATLVCLATGFYPDHVELSWWVNGKEVHSGVSTDPQPLKEQPALNDSRYCLSSRLRVSATFWQNPRNHFRCQVQFYGLSENDEWTQDRAKPVTQIVSAEAWGRADCGFTSESYQQGVLSATILYEILLGKATLYAVLVSALVLMAMVKRKDSRG

SEQ ID NO: 19 - protein, 309 aa, Homo sapiens
MGPGLLCWVLLCLLGAGPVDAGVTQSPTHLIKTRGQHVTLRCSPISGHKSVSWYQQVLGQGPQFIFQYYEKEERGRGNFPDRFSARQFPNYSSELNVNALLLGDSALYLCASSFDVGLPPLHFGNGTRLTVTEDLNKVFPPEVAVFEPSEAEISHTQKATLVCLATGFFPDHVELSWWVNGKEVHSGVSTDPQPLKEQPALNDSRYCLSSRLRVSATFWQNPRNHFRCQVQFYGLSENDEWTQDRAKPVTQIVSAEAWGRADCGFTSVSYQQGVLSATILYEILLGKATLYAVLVSALVLMAMVKRKDF

SEQ ID NO: 20 - protein, 308 aa, Homo sapiens
MGSWTLCCVSLCILVAKHTDAGVIQSPRHEVTEMGQEVTLRCKPISGHDYLFWYRQTMMRGLELLIYFNNNVPIDDSGMPEDRFSAKMPNASFSTLKIQPSEPRDSAVYFCASSYRGTEAFFGQGTRLTVVEDLNKVFPPEVAVFEPSEAEISHTQKATLVCLATGFFPDHVELSWWVNGKEVHSGVSTDPQPLKEQPALNDSRYCLSSRLRVSATFWQNPRNHFRCQVQFYGLSENDEWTQDRAKPVTQIVSAEAWGRADCGFTSVSYQQGVLSATILYEILLGKATLYAVLVSALVLMAMVKRKDF

SEQ ID NO: 21 - protein, 311 aa, Homo sapiens
MGIRLLCRVAFCFLAVGLVDVKVTQSSRYLVKRTGEKVFLECVQDMDHENMFWYRQDPGLGLRLIYFSYDVKMKEKGDIPEGYSVSREKKERFSLILESASTNQTSMYLCASSLGATGANEKLFFGSGTQLSVLEDLNKVFPPEVAVFEPSEAEISHTQKATLVCLATGFFPDHVELSWWVNGKEVHSGVSTDPQPLKEQPALNDSRYCLSSRLRVSATFWQNPRNHFRCQVQFYGLSENDEWTQDRAKPVTQIVSAEAWGRADCGFTSVSYQQGVLSATILYEILLGKATLYAVLVSALVLMAMVKRKDF

SEQ ID NO: 22 - protein, 311 aa, Homo sapiens
MLSLLLLLLGLGSVFSAVISQKPSRDICQRGTSLTIQCQVDSQVTMMFWYRQQPGQSLTLIATANQGSEATYESGFVIDKFPISRPNLTFSTLTVSNMSPEDSSIYLCSVGAGQGPYTDTQYFGPGTRLTVLEDLKNVFPPEVAVFEPSEAEISHTQKATLVCLATGFYPDHVELSWWVNGKEVHSGVSTDPQPLKEQPALNDSRYCLSSRLRVSATFWQNPRNHFRCQVQFYGLSENDEWTQDRAKPVTQIVSAEAWGRADCGFTSESYQQGVLSATILYEILLGKATLYAVLVSALVLMAMVKRKDSRG

SEQ ID NO: 23 - protein, 312 aa, Homo sapiens
MSIGLLCCVAFSLLWASPVNAGVTQTPKFQVLKTGQSMTLQCAQDMNHNSMYWYRQDPGMGLRLIYYSASEGTTDKGEVPNGYNVSRLNKREFSLRLESAAPSQTSVYFCASSEVTGGYNEQFFGPGTRLTVLEDLKNVFPPEVAVFEPSEAEISHTQKATLVCLATGFYPDHVELSWWVNGKEVHSGVSTDPQPLKEQPALNDSRYCLSSRLRVSATFWQNPRNHFRCQVQFYGLSENDEWTQDRAKPVTQIVSAEAWGRADCGFTSESYQQGVLSATILYEILLGKATLYAVLVSALVLMAMVKRKDSRG

SEQ ID NO: 24 - protein, 307 aa, homo sapiens
MLSLLLLLLGLGSVFSAVISQKPSRDICQRGTSLTIQCQVDSQVTMMFWYRQQPGQSLTLIATANQGSEATYESGFVIDKFPISRPNLTFSTLTVSNMSPEDSSIYLCSVEGRGYEQYFGPGTRLTVTEDLKNVFPPEVAVFEPSEAEISHTQKATLVCLATGFYPDHVELSWWVNGKEVHSGVSTDPQPLKEQPALNDSRYCLSSRLRVSATFWQNPRNHFRCQVQFYGLSENDEWTQDRAKPVTQIVSAEAWGRADCGFTSESYQQGVLSATILYEILLGKATLYAVLVSALVLMAMVKRKDSRG

SEQ ID NO: 25 - protein, 310 aa, Homo sapiens
MQWALAVLLAFLSPASQKSSNLEGRTKSVIRQTGSSAEITCDLAEGSTGYIHWYLHQEGKAPQRLLYYDSYTSSVVLESGISPGKYDTYGSTRKNLRMILRNLIENDSGVYYCATWETQELGKKIKVFGPGTKLIITDKQLDADVSPKPTIFLPSIAETKLQKAGTYLCLLEKFFPDVIKIHWQEKKSNTILGSQEGNTMKTNDTYMKFSWLTVPEKSLDKEHRCIVRHENNKNGVDQEIIFPPIKTDVITMDPKDNCSKDANDTLLLQLTNTSAYYMYLLLLLKSVVYFAIITCCLLRRTAFCCNGEKS

SEQ ID NO: 26 - protein, 295 aa, Homo sapiens
MLFSSLLCVFVAFSYSGSSVAQKVTQAQSSVSMPVRKAVTLNCLYETSWWSYYIFWYKQLPSKEMIFLIRQGSDEQNAKSGRYSVNFKKAVKSVALTISALQLEDSAKYFCALGVQALLPILGDTTDKLIFGKGTRVTVEPRSQPHTKPSVFVMKNGTNVACLVKEFYPKDIRINLVSSKKITEFDPAIVISPSGKYNAVKLGKYEDSNSVTCSVQHDNKTVHSTDFEVKTDSTDHVKPKETENTKQPSKSCHKPKAIVHTEKVNMMSLTVLGLRMLFAKTVAVNFLLTAKLFFL

SEQ ID NO: 27 - DNA, 801 bp, Homo sapiens
atgtggggagttttccttctttatgtttccatgaagatgggaggcactacaggacaaaacattgaccagcccactgagatgacagctacggaaggtgccattgtccagatcaactgcacgtaccagacatctgggttcaacgggctgttctggtaccagcaacatgctggcgaagcacccacatttctgtcttacaatgttctggatggtttggaggagaaaggtcgtttttcttcattccttagtcggtctaaagggtacagttacctccttttgaaggagctccagatgaaagactctgcctcttacctctgtgctgtgatggatagcagctataaattgatcttcgggagtgggaccagactgctggtcaggcctgatatccagaaccctgaccctgccgtgtaccagctgagagactctaaatccagtgacaagtctgtctgcctattcaccgattttgattctcaaacaaatgtgtcacaaagtaaggattctgatgtgtatatcacagacaaaactgtgctagacatgaggtctatggacttcaagagcaacagtgctgtggcctggagcaacaaatctgactttgcatgtgcaaacgccttcaacaacagcattattccagaagacaccttcttccccagcccagaaagttcctgtgatgtcaagctggtcgagaaaagctttgaaacagatacgaacctaaactttcaaaacctgtcagtgattgggttccgaatcctcctcctgaaagtggccgggtttaatctgctcatgacgctgcggctgtggtccagc

SEQ ID NO: 28 - DNA, 813 bp, Homo sapiens
atgctactcatcacatcaatgttggtcttatggatgcaattgtcacaggtgaatggacaacaggtaatgcaaattcctcagtaccagcatgtacaagaaggagaggacttcaccacgtactgcaattcctcaactactttaagcaatatacagtggtataagcaaaggcctggtggacatcccgtttttttgatacagttagtgaagagtggagaagtgaagaagcagaaaagactgacatttcagtttggagaagcaaaaaagaacagctccctgcacatcacagccacccagactacagatgtaggaacctacttctgtgcggctgctggtggtactagctatggaaagctgacatttggacaagggaccatcttgactgtccatccaaatatccagaaccctgaccctgccgtgtaccagctgagagactctaaatccagtgacaagtctgtctgcctattcaccgattttgattctcaaacaaatgtgtcacaaagtaaggattctgatgtgtatatcacagacaaaactgtgctagacatgaggtctatggacttcaagagcaacagtgctgtggcctggagcaacaaatctgactttgcatgtgcaaacgccttcaacaacagcattattccagaagacaccttcttccccagcccagaaagttcctgtgatgtcaagctggtcgagaaaagctttgaaacagatacgaacctaaactttcaaaacctgtcagtgattgggttccgaatcctcctcctgaaagtggccgggtttaatctgctcatgacgctgcggctgtggtccagc

SEQ ID NO: 29 - DNA, 830 bp, Homo sapiens
atgaagacatttgctggattttcgttcctgtttttgtggctgcagctggactgtatgagtagaggagaggatgtggagcagagtcttttcctgagtgtccgagagggagacagctccgttataaactgcacttacacagacagctcctccacctacttatactggtataagcaagaacctggagcaggtctccagttgctgacgtatattttttcaaatatggacatgaaacaagaccaaagactcactgttctattgaataaaaaggataaacatctgtctctgcgcattgcagacacccagactggggactcagctatctacttctgtgcagagacctggaccgacagaggctcaaccctggggaggctatactttggaagaggaactcagttgactgtctggcctgatatccagaaccctgaccctgccgtgtaccagctgagagactctaaatccagtgacaagtctgtctgcctattcaccgattttgattctcaaacaaatgtgtcacaaagtaaggattctgatgtgtatatcacagacaaaactgtgctagacatgaggtctatggacttcaagagcaacagtgctgtggcctggagcaacaaatctgactttgcatgtgcaaacgccttcaacaacagcattattccagaagacaccttcttccccagcccagaaagttcctgtgatgtcaagctggtcgagaaaagctttgaaacagatacgaacctaaactttcaaaacctgtcagtgattgggttccgaatcctcctcctgaaagtggccgggtttaatctgctcatgacgttgcggctgtggtccag

SEQ ID NO: 30 - DNA, 840 bp, Homo sapiens
atggccatgctcctgggggcatcagtgctgattctgtggcttcagacagactgggtaaacagtcaacagaagaatgatgaccagcaagttaagcaaaattcaccatccctgagcgtccaggaaggaagaatttctattctgaactgtgactatactaacagcatgtttgattatttcctatggtacaaaaaataccctgctgaaggtcctacattcctgatatctataagttccattaaggataaaaatgaagatggaagattcactgtcttcttaaacaaaagtgccaagcacctctctctgcacattgtgccctcccagcctggagactctgcagtgtacttctgtgcagcaagtctttataaccagggaggaaagcttatcttcggacagggaacggagttatctgtgaaacccaatatccagaaccctgaccctgccgtgtaccagctgagagactctaaatccagtgacaagtctgtctgcctattcaccgattttgattctcaaacaaatgtgtcacaaagtaaggattctgatgtgtatatcacagacaaaactgtgctagacatgaggtctatggacttcaagagcaacagtgctgtggcctggagcaacaaatctgactttgcatgtgcaaacgccttcaacaacagcattattccagaagacaccttcttccccagcccagaaagttcctgtgatgtcaagctggtcgagaaaagctttgaaacagatacgaacctaaactttcaaaacctgtcagtgattgggttccgaatcctcctcctgaaagtggccgggtttaatctgctcatgacgctgcggctgtggtccagc

SEQ ID NO: 31 - DNA, 822 bp, Homo sapiens
atggagaagaatcctttggcagccccattactaatcctctggtttcatcttgactgcgtgagcagcatactgaacgtggaacaaagtcctcagtcactgcatgttcaggagggagacagcaccaatttcacctgcagcttcccttccagcaatttttatgccttacactggtacagatgggaaactgcaaaaagccccgaggccttgtttgtaatgactttaaatggggatgaaaagaagaaaggacgaataagtgccactcttaataccaaggagggttacagctatttgtacatcaaaggatcccagcctgaagactcagccacatacctctgtgcctcgggggattccgggtatgcactcaacttcggcaaaggcacctcgctgttggtcacaccccatatccagaaccctgaccctgccgtgtaccagctgagagactctaaatccagtgacaagtctgtctgcctattcaccgattttgattctcaaacaaatgtgtcacaaagtaaggattctgatgtgtatatcacagacaaaactgtgctagacatgaggtctatggacttcaagagcaacagtgctgtggcctggagcaacaaatctgactttgcatgtgcaaacgccttcaacaacagcattattccagaagacaccttcttccccagcccagaaagttcctgtgatgtcaagctggtcgagaaaagctttgaaacagatacgaacctaaactttcaaaacctgtcagtgattgggttccgaatcctcctcctgaaagtggccgggtttaatctgctcatgacgctgcggctgtggtccagc

SEQ ID NO: 32 - DNA, 828 bp, Homo sapiens
atgaactattctccaggcttagtatctctgatactcttactgcttggaagaacccgtggaaattcagtgacccagatggaagggccagtgactctctcagaagaggccttcctgactataaactgcacgtacacagccacaggatacccttcccttttctggtatgtccaatatcctggagaaggtctacagctcctcctgaaagccacgaaggctgatgacaagggaagcaacaaaggttttgaagccacataccgtaaagaaaccacttctttccacttggagaaaggctcagttcaagtgtcagactcagcggtgtacttctgtgctctgacaatatgggattatggaggaagccaaggaaatctcatctttggaaaaggcactaaactctctgttaaaccaaatatccagaaccctgaccctgccgtgtaccagctgagagactctaaatccagtgacaagtctgtctgcctattcaccgattttgattctcaaacaaatgtgtcacaaagtaaggattctgatgtgtatatcacagacaaaactgtgctagacatgaggtctatggacttcaagagcaacagtgctgtggcctggagcaacaaatctgactttgcatgtgcaaacgccttcaacaacagcattattccagaagacaccttcttccccagcccagaaagttcctgtgatgtcaagctggtcgagaaaagctttgaaacagatacgaacctaaactttcaaaacctgtcagtgattgggttccgaatcctcctcctgaaagtggccgggtttaatctgctcatgacgctgcggctgtggtccagc

SEQ ID NO: 33 - DNA, 807 bp, Homo sapiens
atggtcctgaaattctccgtgtccattctttggattcagttggcatgggtgagcacccagctgctggagcagagccctcagtttctaagcatccaagagggagaaaatctcactgtgtactgcaactcctcaagtgttttttccagcttacaatggtacagacaggagcctggggaaggtcctgtcctcctggtgacagtagttacgggtggagaagtgaagaagctgaagagactaacctttcagtttggtgatgcaagaaaggacagttctctccacatcactgcagcccagcctggtgatacaggcctctacctctgtgcaggagaaaattccgggtatgcactcaacttcggcaaaggcacctcgctgttggtcacaccccatatccagaaccctgaccctgccgtgtaccagctgagagactctaaatccagtgacaagtctgtctgcctattcaccgattttgattctcaaacaaatgtgtcacaaagtaaggattctgatgtgtatatcacagacaaaactgtgctagacatgaggtctatggacttcaagagcaacagtgctgtggcctggagcaacaaatctgactttgcatgtgcaaacgccttcaacaacagcattattccagaagacaccttcttccccagcccagaaagttcctgtgatgtcaagctggtcgagaaaagctttgaaacagatacgaacctaaactttcaaaacctgtcagtgattgggttccgaatcctcctcctgaaagtggccgggtttaatctgctcatgacgctgcggctgtggtccagc

SEQ ID NO: 34 - DNA, 825 bp, Homo sapiens
atgatgaaatccttgagagttttactggtgatcctgtggcttcagttaagctgggtttggagccaacagaaggaggtggagcaggatcctggaccactcagtgttccagagggagccattgtttctctcaactgcacttacagcaacagtgcttttcaatacttcatgtggtacagacagtattccagaaaaggccctgagttgctgatgtacacatactccagtggtaacaaagaagatggaaggtttacagcacaggtcgataaatccagcaagtatatctccttgttcatcagagactcacagcccagtgattcagccacctacctctgtgcaatgagcctatcaggaggaagctacatacctacatttggaagaggaaccagccttattgttcatccgtatatccagaaccctgaccctgccgtgtaccagctgagagactctaaatccagtgacaagtctgtctgcctattcaccgattttgattctcaaacaaatgtgtcacaaagtaaggattctgatgtgtatatcacagacaaaactgtgctagacatgaggtctatggacttcaagagcaacagtgctgtggcctggagcaacaaatctgactttgcatgtgcaaacgccttcaacaacagcattattccagaagacaccttcttccccagcccagaaagttcctgtgatgtcaagctggtcgagaaaagctttgaaacagatacgaacctaaactttcaaaacctgtcagtgattgggttccgaatcctcctcctgaaagtggccgggtttaatctgctcatgacgctgcggctgtggtccagc

SEQ ID NO: 35 - DNA, 825 bp, Homo sapiens
atgctccttgaacatttattaataatcttgtggatgcagctgacatgggtcagtggtcaacagctgaatcagagtcctcaatctatgtttatccaggaaggagaagatgtctccatgaactgcacttcttcaagcatatttaacacctggctatggtacaagcaggaccctggggaaggtcctgtcctcttgatagccttatataaggctggtgaattgacctcaaatggaagactgactgctcagtttggtataaccagaaaggacagcttcctgaatatctcagcatccatacctagtgatgtaggcatctacttctgtgctgggcagctaggaggggctggtggtactagctatggaaagctgacatttggacaagggaccatcttgactgtccatccaaatatccagaaccctgaccctgccgtgtaccagctgagagactctaaatccagtgacaagtctgtctgcctattcaccgattttgattctcaaacaaatgtgtcacaaagtaaggattctgatgtgtatatcacagacaaaactgtgctagacatgaggtctatggacttcaagagcaacagtgctgtggcctggagcaacaaatctgactttgcatgtgcaaacgccttcaacaacagcattattccagaagacaccttcttccccagcccagaaagttcctgtgatgtcaagctggtcgagaaaagctttgaaacagatacgaacctaaactttcaaaacctgtcagtgattgggttccgaatcctcctcctgaaagtggccgggtttaatctgctcatgacgctgcggctgtggtccagc

SEQ ID NO: 36 - DNA, 822 bp, Homo sapiens
atgacatccattcgagctgtatttatattcctgtggctgcagctggacttggtgaatggagagaatgtggagcagcatccttcaaccctgagtgtccaggagggagacagcgctgttatcaagtgtacttattcagacagtgcctcaaactacttcccttggtataagcaagaacttggaaaaggacctcagcttattatagacattcgttcaaatgtgggcgaaaagaaagaccaacgaattgctgttacattgaacaagacagccaaacatttctccctgcacatcacagagacccaacctgaagactcggctgtctacttctgtgcagcaaactggagcccgcaaggaaatgagaaattaacctttgggactggaacaagactcaccatcatacccaatatccagaaccctgaccctgccgtgtaccagctgagagactctaaatccagtgacaagtctgtctgcctattcaccgattttgattctcaaacaaatgtgtcacaaagtaaggattctgatgtgtatatcacagacaaaactgtgctagacatgaggtctatggacttcaagagcaacagtgctgtggcctggagcaacaaatctgactttgcatgtgcaaacgccttcaacaacagcattattccagaagacaccttcttccccagcccagaaagttcctgtgatgtcaagctggtcgagaaaagctttgaaacagatacgaacctaaactttcaaaacctgtcagtgattgggttccgaatcctcctcctgaaagtggccgggtttaatctgctcatgacgctgcggctgtggtccagc

SEQ ID NO: 37 - DNA, 801 bp, Homo sapiens
atgtggggagttttccttctttatgtttccatgaagatgggaggcactacaggacaaaacattgaccagcccactgagatgacagctacggaaggtgccattgtccagatcaactgcacgtaccagacatctgggttcaacgggctgttctggtaccagcaacatgctggcgaagcacccacatttctgtcttacaatgttctggatggtttggaggagaaaggtcgtttttcttcattccttagtcggtctaaagggtacagttacctccttttgaaggagctccagatgaaagactctgcctcttacctctgtgcttccatggatagcaactatcagttaatctggggcgctgggaccaagctaattataaagccagatatccagaaccctgaccctgccgtgtaccagctgagagactctaaatccagtgacaagtctgtctgcctattcaccgattttgattctcaaacaaatgtgtcacaaagtaaggattctgatgtgtatatcacagacaaaactgtgctagacatgaggtctatggacttcaagagcaacagtgctgtggcctggagcaacaaatctgactttgcatgtgcaaacgccttcaacaacagcattattccagaagacaccttcttccccagcccagaaagttcctgtgatgtcaagctggtcgagaaaagctttgaaacagatacgaacctaaactttcaaaacctgtcagtgattgggttccgaatcctcctcctgaaagtggccgggtttaatctgctcatgacgctgcggctgtggtccagc

SEQ ID NO: 38 - DNA, 822 bp, Homo sapiens
atgatatccttgagagttttactggtgatcctgtggcttcagttaagctgggtttggagccaacggaaggaggtggagcaggatcctggacccttcaatgttccagagggagccactgtcgctttcaactgtacttacagcaacagtgcttctcagtctttcttctggtacagacaggattgcaggaaagaacctaagttgctgatgtccgtatactccagtggtaatgaagatggaaggtttacagcacagctcaatagagccagccagtatatttccctgctcatcagagactccaagctcagtgattcagccacctacctctgtgtggtgaacagattcacaagggatggaaacaaactggtctttggcgcaggaaccattctgagagtcaagtcctatatccagaaccctgaccctgccgtgtaccagctgagagactctaaatccagtgacaagtctgtctgcctattcaccgattttgattctcaaacaaatgtgtcacaaagtaaggattctgatgtgtatatcacagacaaaactgtgctagacatgaggtctatggacttcaagagcaacagtgctgtggcctggagcaacaaatctgactttgcatgtgcaaacgccttcaacaacagcattattccagaagacaccttcttccccagcccagaaagttcctgtgatgtcaagctggtcgagaaaagctttgaaacagatacgaacctaaactttcaaaacctgtcagtgattgggttccgaatcctcctcctgaaagtggccgggtttaatctgctcatgacgctgcggctgtggtccagc

SEQ ID NO: 39 - DNA, 942 bp, Homo sapiens
atgctgctgcttctgctgcttctggggccaggctccgggcttggtgctgtcgtctctcaacatccgagctgggttatctgtaagagtggaacctctgtgaagatcgagtgccgttccctggactttcaggccacaactatgttttggtatcgtcagttcccgaaacagagtctcatgctgatggcaacttccaatgagggctccaaggccacatacgagcaaggcgtcgagaaggacaagtttctcatcaaccatgcaagcctgaccttgtccactctgacagtgaccagtgcccatcctgaagacagcagcttctacatctgcagtgcgaaggtgactagcgggcaacaccaagggaccacagatacgcagtattttggcccaggcacccggctgacagtgctcgaggacctgaaaaacgtgttcccacccgaggtcgctgtgtttgagccatcagaagcagagatctcccacacccaaaaggccacactggtgtgcctggccacaggcttctaccccgaccacgtggagctgagctggtgggtgaatgggaaggaggtgcacagtggggtcagcacagacccgcagcccctcaaggagcagcccgccctcaatgactccagatactgcctgagcagccgcctgagggtctcggccaccttctggcagaacccccgcaaccacttccgctgtcaagtccagttctacgggctctcggagaatgacgagtggacccaggatagggccaaacctgtcacccagatcgtcagcgccgaggcctggggtagagcagactgtggcttcacctccgagtcttaccagcaaggggtcctgtctgccaccatcctctatgagatcttgctagggaaggccaccttgtatgccgtgctggtcagtgccctcgtgctgatggccatggtcaagagaaaggattccagaggc

SEQ ID NO: 40 - DNA, 933 bp, Homo sapiens
atgactatcaggctcctctgctacatgggcttttattttctgggggcaggcctcatggaagctgacatctaccagaccccaagataccttgttatagggacaggaaagaagatcactctggaatgttctcaaaccatgggccatgacaaaatgtactggtatcaacaagatccaggaatggaactacacctcatccactattcctatggagttaattccacagagaagggagatctttcctctgagtcaacagtctccagaataaggacggagcattttcccctgaccctggagtctgccaggccctcacatacctctcagtacctctgtgccagcagtgaatatatccagtactctggaaacaccatatattttggagagggaagttggctcactgttgtagaggacctgaacaaggtgttcccacccgaggtcgctgtgtttgagccatcagaagcagagatctcccacacccaaaaggccacactggtgtgcctggccacaggcttcttccctgaccacgtggagctgagctggtgggtgaatgggaaggaggtgcacagtggggtcagcacggacccgcagcccctcaaggagcagcccgccctcaatgactccagatactgcctgagcagccgcctgagggtctcggccaccttctggcagaacccccgcaaccacttccgctgtcaagtccagttctacgggctctcggagaatgacgagtggacccaggatagggccaaacccgtcacccagatcgtcagcgccgaggcctggggtagagcagactgtggctttacctcggtgtcctaccagcaaggggtcctgtctgccaccatcctctatgagatcctgctagggaaggccaccctgtatgctgtgctggtcagcgcccttgtgttgatggccatggtcaagagaaaggatttc

SEQ ID NO: 41 - DNA, 936 bp, Homo sapiens
atgggcttcaggctcctctgctgtgtggccttttgtctcctgggagcaggcccagtggattctggagtcacacaaaccccaaagcacctgatcacagcaactggacagcgagtgacgctgagatgctcccctaggtctggagacctctctgtgtactggtaccaacagagcctggaccagggcctccagttcctcattcagtattataatggagaagagagagcaaaaggaaacattcttgaacgattctccgcacaacagttccctgacttgcactctgaactaaacctgagctctctggagctgggggactcagctttgtatttctgtgccagcagcgtcggagggggattggcagatacgcagtattttggcccaggcacccggctgacagtgctcgaggacctgaaaaacgtgttcccacccgaggtcgctgtgtttgagccatcagaagcagagatctcccacacccaaaaggccacactggtgtgcctggccacaggcttctaccccgaccacgtggagctgagctggtgggtgaatgggaaggaggtgcacagtggggtcagcacagacccgcagcccctcaaggagcagcccgccctcaatgactccagatactgcctgagcagccgcctgagggtctcggccaccttctggcagaacccccgcaaccacttccgctgtcaagtccagttctacgggctctcggagaatgacgagtggacccaggatagggccaaacctgtcacccagatcgtcagcgccgaggcctggggtagagcagactgtggcttcacctccgagtcttaccagcaaggggtcctgtctgccaccatcctctatgagatcttgctagggaaggccaccttgtatgccgtgctggtcagtgccctcgtgctgatggccatggtcaagagaaaggattccagaggc

SEQ ID NO: 42 - DNA, 939 bp, Homo sapiens
atgagcatcggcctcctgtgctgtgcagccttgtctctcctgtgggcaggtccagtgaatgctggtgtcactcagaccccaaaattccaggtcctgaagacaggacagagcatgacactgcagtgtgcccaggatatgaaccatgaatacatgtcctggtatcgacaagacccaggcatggggctgaggctgattcattactcagttggtgctggtatcactgaccaaggagaagtccccaatggctacaatgtctccagatcaaccacagaggatttcccgctcaggctgctgtcggctgctccctcccagacatctgtgtacttctgtgccagcggaatcagcgggacagcgagctcctataattcacccctccactttgggaacgggaccaggctcactgtgacagaggacctgaacaaggtgttcccacccgaggtcgctgtgtttgagccatcagaagcagagatctcccacacccaaaaggccacactggtgtgcctggccacaggcttcttccctgaccacgtggagctgagctggtgggtgaatgggaaggaggtgcacagtggggtcagcacggacccgcagcccctcaaggagcagcccgccctcaatgactccagatactgcctgagcagccgcctgagggtctcggccaccttctggcagaacccccgcaaccacttccgctgtcaagtccagttctacgggctctcggagaatgacgagtggacccaggatagggccaaacccgtcacccagatcgtcagcgccgaggcctggggtagagcagactgtggctttacctcggtgtcctaccagcaaggggtcctgtctgccaccatcctctatgagatcctgctagggaaggccaccctgtatgctgtgctggtcagcgcccttgtgttgatggccatggtcaagagaaaggatttc

SEQ ID NO: 43 - DNA, 927 bp, Homo sapiens
atgggtcctgggcttctccactggatggccctttgtctccttggaacaggtcatggggatgccatggtcatccagaacccaagataccaggttacccagtttggaaagccagtgaccctgagttgttctcagactttgaaccataacgtcatgtactggtaccagcagaagtcaagtcaggccccaaagctgctgttccactactatgacaaagattttaacaatgaagcagacacccctgataacttccaatccaggaggccgaacacttctttctgctttcttgacatccgctcaccaggcctgggggacgcagccatgtacctgtgtgccaccagcagagagtgggagacccagtacttcgggccaggcacgcggctcctggtgctcgaggacctgaaaaacgtgttcccacccgaggtcgctgtgtttgagccatcagaagcagagatctcccacacccaaaaggccacactggtgtgcctggccacaggcttctaccccgaccacgtggagctgagctggtgggtgaatgggaaggaggtgcacagtggggtcagcacagacccgcagcccctcaaggagcagcccgccctcaatgactccagatactgcctgagcagccgcctgagggtctcggccaccttctggcagaacccccgcaaccacttccgctgtcaagtccagttctacgggctctcggagaatgacgagtggacccaggatagggccaaacctgtcacccagatcgtcagcgccgaggcctggggtagagcagactgtggcttcacctccgagtcttaccagcaaggggtcctgtctgccaccatcctctatgagatcttgctagggaaggccaccttgtatgccgtgctggtcagtgccctcgtgctgatggccatggtcaagagaaaggattccagaggc

SEQ ID NO: 44 - DNA, 945 bp, Homo sapiens
atgactatcaggctcctctgctacatgggcttttattttctgggggcaggcctcatggaagctgacatctaccagaccccaagataccttgttatagggacaggaaagaagatcactctggaatgttctcaaaccatgggccatgacaaaatgtactggtatcaacaagatccaggaatggaactacacctcatccactattcctatggagttaattccacagagaagggagatctttcctctgagtcaacagtctccagaataaggacggagcattttcccctgaccctggagtctgccaggccctcacatacctctcagtacctctgtgccagcagccaactttaccgggacacctcgaacaccggggagctgttttttggagaaggctctaggctgaccgtactggaggacctgaaaaacgtgttcccacccgaggtcgctgtgtttgagccatcagaagcagagatctcccacacccaaaaggccacactggtgtgcctggccacaggcttctaccccgaccacgtggagctgagctggtgggtgaatgggaaggaggtgcacagtggggtcagcacagacccgcagcccctcaaggagcagcccgccctcaatgactccagatactgcctgagcagccgcctgagggtctcggccaccttctggcagaacccccgcaaccacttccgctgtcaagtccagttctacgggctctcggagaatgacgagtggacccaggatagggccaaacctgtcacccagatcgtcagcgccgaggcctggggtagagcagactgtggcttcacctccgagtcttaccagcaaggggtcctgtctgccaccatcctctatgagatcttgctagggaaggccaccttgtatgccgtgctggtcagtgccctcgtgctgatggccatggtcaagagaaaggattccagaggc

SEQ ID NO: 45 - DNA, 927 bp, Homo sapiens
atgggccctgggctcctctgctgggtgctgctttgtctcctgggagcaggcccagtggacgctggagtcacccaaagtcccacacacctgatcaaaacgagaggacagcacgtgactctgagatgctctcctatctctgggcacaagagtgtgtcctggtaccaacaggtcctgggtcaggggccccagtttatctttcagtattatgagaaagaagagagaggaagaggaaacttccctgatcgattctcagctcgccagttccctaactatagctctgagctgaatgtgaacgccttgttgctgggggactcggccctgtatctctgtgccagcagctttgacgttggtttgccacccctccactttgggaacgggaccaggctcactgtgacagaggacctgaacaaggtgttcccacccgaggtcgctgtgtttgagccatcagaagcagagatctcccacacccaaaaggccacactggtgtgcctggccacaggcttcttccctgaccacgtggagctgagctggtgggtgaatgggaaggaggtgcacagtggggtcagcacggacccgcagcccctcaaggagcagcccgccctcaatgactccagatactgcctgagcagccgcctgagggtctcggccaccttctggcagaacccccgcaaccacttccgctgtcaagtccagttctacgggctctcggagaatgacgagtggacccaggatagggccaaacccgtcacccagatcgtcagcgccgaggcctggggtagagcagactgtggctttacctcggtgtcctaccagcaaggggtcctgtctgccaccatcctctatgagatcctgctagggaaggccaccctgtatgctgtgctggtcagcgcccttgtgttgatggccatggtcaagagaaaggatttc

SEQ ID NO: 46 - DNA, 924 bp, Homo sapiens
atgggctcctggaccctctgctgtgtgtccctttgcatcctggtagcaaagcacacagatgctggagttatccagtcaccccggcacgaggtgacagagatgggacaagaagtgactctgagatgtaaaccaatttcaggacacgactaccttttctggtacagacagaccatgatgcggggactggagttgctcatttactttaacaacaacgttccgatagatgattcagggatgcccgaggatcgattctcagctaagatgcctaatgcatcattctccactctgaagatccagccctcagaacccagggactcagctgtgtacttctgtgccagcagctacaggggcactgaagctttctttggacaaggcaccagactcacagttgtagaggacctgaacaaggtgttcccacccgaggtcgctgtgtttgagccatcagaagcagagatctcccacacccaaaaggccacactggtgtgcctggccacaggcttcttccctgaccacgtggagctgagctggtgggtgaatgggaaggaggtgcacagtggggtcagcacggacccgcagcccctcaaggagcagcccgccctcaatgactccagatactgcctgagcagccgcctgagggtctcggccaccttctggcagaacccccgcaaccacttccgctgtcaagtccagttctacgggctctcggagaatgacgagtggacccaggatagggccaaacccgtcacccagatcgtcagcgccgaggcctggggtagagcagactgtggctttacctcggtgtcctaccagcaaggggtcctgtctgccaccatcctctatgagatcctgctagggaaggccaccctgtatgctgtgctggtcagcgcccttgtgttgatggccatggtcaagagaaaggatttc

SEQ ID NO: 47 - DNA, 933 bp, Homo sapiens
atgggaatcaggctcctgtgtcgtgtggccttttgtttcctggctgtaggcctcgtagatgtgaaagtaacccagagctcgagatatctagtcaaaaggacgggagagaaagtttttctggaatgtgtccaggatatggaccatgaaaatatgttctggtatcgacaagacccaggtctggggctacggctgatctatttctcatatgatgttaaaatgaaagaaaaaggagatattcctgaggggtacagtgtctctagagagaagaaggagcgcttctccctgattctggagtccgccagcaccaaccagacatctatgtacctctgtgccagcagcttaggggcgacaggggctaatgaaaaactgttttttggcagtggaacccagctctctgtcttggaggacctgaacaaggtgttcccacccgaggtcgctgtgtttgagccatcagaagcagagatctcccacacccaaaaggccacactggtgtgcctggccacaggcttcttccctgaccacgtggagctgagctggtgggtgaatgggaaggaggtgcacagtggggtcagcacggacccgcagcccctcaaggagcagcccgccctcaatgactccagatactgcctgagcagccgcctgagggtctcggccaccttctggcagaacccccgcaaccacttccgctgtcaagtccagttctacgggctctcggagaatgacgagtggacccaggatagggccaaacccgtcacccagatcgtcagcgccgaggcctggggtagagcagactgtggctttacctcggtgtcctaccagcaaggggtcctgtctgccaccatcctctatgagatcctgctagggaaggccaccctgtatgctgtgctggtcagcgcccttgtgttgatggccatggtcaagagaaaggatttc

SEQ ID NO: 48 - DNA, 933 bp, Homo sapiens
atgctgagtcttctgctccttctcctgggactaggctctgtgttcagtgctgtcatctctcaaaagccaagcagggatatctgtcaacgtggaacctccctgacgatccagtgtcaagtcgatagccaagtcaccatgatgttctggtaccgtcagcaacctggacagagcctgacactgatcgcaactgcaaatcagggctctgaggccacatatgagagtggatttgtcattgacaagtttcccatcagccgcccaaacctaacattctcaactctgactgtgagcaacatgagccctgaagacagcagcatatatctctgcagcgttggggcggggcaaggaccttacacagatacgcagtattttggcccaggcacccggctgacagtgctcgaggacctgaaaaacgtgttcccacccgaggtcgctgtgtttgagccatcagaagcagagatctcccacacccaaaaggccacactggtgtgcctggccacaggcttctaccccgaccacgtggagctgagctggtgggtgaatgggaaggaggtgcacagtggggtcagcacagacccgcagcccctcaaggagcagcccgccctcaatgactccagatactgcctgagcagccgcctgagggtctcggccaccttctggcagaacccccgcaaccacttccgctgtcaagtccagttctacgggctctcggagaatgacgagtggacccaggatagggccaaacctgtcacccagatcgtcagcgccgaggcctggggtagagcagactgtggcttcacctccgagtcttaccagcaaggggtcctgtctgccaccatcctctatgagatcttgctagggaaggccaccttgtatgccgtgctggtcagtgccctcgtgctgatggccatggtcaagagaaaggattccagaggc

SEQ ID NO: 49 - DNA, 936 bp, Homo sapiens
atgagcatcggcctcctgtgctgtgtggccttttctctcctgtgggcaagtccagtgaatgctggtgtcactcagaccccaaaattccaggtcctgaagacaggacagagcatgacactgcagtgtgcccaggatatgaaccataactccatgtactggtatcgacaagacccaggcatgggactgaggctgatttattactcagcttctgagggtaccactgacaaaggagaagtccccaatggctacaatgtctccagattaaacaaacgggagttctcgctcaggctggagtcggctgctccctcccagacatctgtgtacttctgtgccagcagtgaggtgacagggggatacaatgagcagttcttcgggccagggacacggctcaccgtgctagaggacctgaaaaacgtgttcccacccgaggtcgctgtgtttgagccatcagaagcagagatctcccacacccaaaaggccacactggtgtgcctggccacaggcttctaccccgaccacgtggagctgagctggtgggtgaatgggaaggaggtgcacagtggggtcagcacagacccgcagcccctcaaggagcagcccgccctcaatgactccagatactgcctgagcagccgcctgagggtctcggccaccttctggcagaacccccgcaaccacttccgctgtcaagtccagttctacgggctctcggagaatgacgagtggacccaggatagggccaaacctgtcacccagatcgtcagcgccgaggcctggggtagagcagactgtggcttcacctccgagtcttaccagcaaggggtcctgtctgccaccatcctctatgagatcttgctagggaaggccaccttgtatgccgtgctggtcagtgccctcgtgctgatggccatggtcaagagaaaggattccagaggc

SEQ ID NO: 50 - DNA, 921 bp, Homo sapiens
atgctgagtcttctgctccttctcctgggactaggctctgtgttcagtgctgtcatctctcaaaagccaagcagggatatctgtcaacgtggaacctccctgacgatccagtgtcaagtcgatagccaagtcaccatgatgttctggtaccgtcagcaacctggacagagcctgacactgatcgcaactgcaaatcagggctctgaggccacatatgagagtggatttgtcattgacaagtttcccatcagccgcccaaacctaacattctcaactctgactgtgagcaacatgagccctgaagacagcagcatatatctctgcagcgttgaaggcaggggttacgagcagtacttcgggccgggcaccaggctcacggtcacagaggacctgaaaaacgtgttcccacccgaggtcgctgtgtttgagccatcagaagcagagatctcccacacccaaaaggccacactggtgtgcctggccacaggcttctaccccgaccacgtggagctgagctggtgggtgaatgggaaggaggtgcacagtggggtcagcacagacccgcagcccctcaaggagcagcccgccctcaatgactccagatactgcctgagcagccgcctgagggtctcggccaccttctggcagaacccccgcaaccacttccgctgtcaagtccagttctacgggctctcggagaatgacgagtggacccaggatagggccaaacctgtcacccagatcgtcagcgccgaggcctggggtagagcagactgtggcttcacctccgagtcttaccagcaaggggtcctgtctgccaccatcctctatgagatcttgctagggaaggccaccttgtatgccgtgctggtcagtgccctcgtgctgatggccatggtcaagagaaaggattccagaggc

SEQ ID NO: 51 - DNA, 930 bp, Homo sapiens
atgcagtgggccctagcggtgcttctagctttcctgtctcctgccagtcagaaatcttccaacttggaagggagaacgaagtcagtcatcaggcagactgggtcatctgctgaaatcacttgtgatcttgctgaaggaagtaccggctacatccactggtacctacaccaggaggggaaggccccacagcgtcttctgtactatgactcctacacctccagcgttgtgttggaatcaggaatcagcccagggaagtatgatacttatggaagcacaaggaagaacttgagaatgatactgcgaaatcttattgaaaatgactctggagtctattactgtgccacctgggaaactcaagagttgggcaaaaaaatcaaggtatttggtcccggaacaaagcttatcattacagataaacaacttgatgcagatgtttcccccaagcccactatttttcttccttcaattgctgaaacaaagctccagaaggctggaacatacctttgtcttcttgagaaatttttccctgatgttattaagatacattggcaagaaaagaagagcaacacgattctgggatcccaggaggggaacaccatgaagactaacgacacatacatgaaatttagctggttaacggtgccagaaaagtcactggacaaagaacacagatgtatcgtcagacatgagaataataaaaacggagttgatcaagaaattatctttcctccaataaagacagatgtcatcacaatggatcccaaagacaattgttcaaaagatgcaaatgatacactactgctgcagctcacaaacacctctgcatattacatgtacctcctcctgctcctcaagagtgtggtctattttgccatcatcacctgctgtctgcttagaagaacggctttctgctgcaatggagagaaatca

SEQ ID NO: 52 - DNA, 885 bp, Homo sapiens
atgctgttctccagcctgctgtgtgtatttgtggccttcagctactctggatcaagtgtggcccagaaggttactcaagcccagtcatcagtatccatgccagtgaggaaagcagtcaccctgaactgcctgtatgaaacaagttggtggtcatattatattttttggtacaagcaacttcccagcaaagagatgattttccttattcgccagggttctgatgaacagaatgcaaaaagtggtcgctattctgtcaacttcaagaaagcagtgaaatccgtcgccttaaccatttcagccttacagctagaagattcagcaaagtacttttgtgctcttggggtccaagccctcctacccatactgggggataccaccgataaactcatctttggaaaaggaacccgtgtgactgtggaaccaagaagtcagcctcataccaaaccatccgtttttgtcatgaaaaatggaacaaatgtcgcttgtctggtgaaggaattctaccccaaggatataagaataaatctcgtgtcatccaagaagataacagagtttgatcctgctattgtcatctctcccagtgggaagtacaatgctgtcaagcttggtaaatatgaagattcaaattcagtgacatgttcagttcaacacgacaataaaactgtgcactccactgactttgaagtgaagacagattctacagatcacgtaaaaccaaaggaaactgaaaacacaaagcaaccttcaaagagctgccataaacccaaagccatagttcataccgagaaggtgaacatgatgtccctcacagtgcttgggctacgaatgctgtttgcaaagactgttgccgtcaattttctcttgactgccaagttatttttcttg

SEQ ID NO: 53 - DNA, 22 bp, Homo sapiens
ctcggcaggccgagccacgggc

SEQ ID NO: 54 - DNA, 22 bp, Homo sapiens
gcccgtggctcggcctgccgag

SEQ ID NO: 55 - DNA, 27 bp, Artificial Sequence
  primer with restriction site
ctcgagatgtctcgctccgtggcctta

SEQ ID NO: 56 - DNA, 32 bp, Artificial Sequence
  primer with restriction site
gtgtgagttttgtcgctagcctgggggacctg

SEQ ID NO: 57 - DNA, 32 bp, Artificial Sequence
  primer with restriction site
caggtcccccaggctagcgacaaaactcacac

SEQ ID NO: 58 - DNA, 31 bp, Artificial Sequence
  primer with restriction site
gcggccgctcatttacccggagacagggaga